European Patent Specification EP 3 878 970 B1, published September 11, 2024. Title: LAMININ 511 PRODUCTION PROMOTER, BASAL EPIDERMAL LAYER STABILIZER AND/OR SCREENING METHOD FOR AGENT TO MINIMIZE REDUCTION IN OR PROMOTE INCREASE IN EPIDERMAL STEM CELLS. Applicant: Shiseido Company, Limited. The sequence listing filed with the application follows.

SEQUENCE LISTING (36 sequences)

SEQ ID NO: 1 - DNA, 20 bp, Artificial Sequence
  Primer
cacggctctgaccgacatag

SEQ ID NO: 2 - DNA, 19 bp, Artificial Sequence
  Primer
cccagccctctacgacagt

SEQ ID NO: 3 - DNA, 22 bp, Artificial Sequence
  Primer
gtgggatcgagacatgtaagca

SEQ ID NO: 4 - DNA, 19 bp, Artificial Sequence
  Primer
caatccaaatgcggcatct

SEQ ID NO: 5 - DNA, 22 bp, Artificial Sequence
  Primer
tggctggattatgtactcgtgg

SEQ ID NO: 6 - DNA, 22 bp, Artificial Sequence
  Primer
ctgtagcacctacttcgtggca

SEQ ID NO: 7 - DNA, 23 bp, Artificial Sequence
  Primer
ctttgtagtctctggcaagatgc

SEQ ID NO: 8 - DNA, 24 bp, Artificial Sequence
  Primer
cgggtataaacttcaactctgtgc

SEQ ID NO: 9 - DNA, 20 bp, Artificial Sequence
  Primer
tccaaggatatatgccccaa

SEQ ID NO: 10 - DNA, 20 bp, Artificial Sequence
  Primer
gaactcggtttctcagcagc

SEQ ID NO: 11 - DNA, 20 bp, Artificial Sequence
  Primer
cttgacctgggttctgggta

SEQ ID NO: 12 - DNA, 20 bp, Artificial Sequence
  Primer
ggccaaaggaacatttgaag

SEQ ID NO: 13 - DNA, 18 bp, Artificial Sequence
  Primer
ttgcagtcaacagtcgaa

SEQ ID NO: 14 - DNA, 19 bp, Artificial Sequence
  Primer
ttctgacgactccttgttc

SEQ ID NO: 15 - DNA, 20 bp, Artificial Sequence
  Primer
ttggaccaagatgtcctgag

SEQ ID NO: 16 - DNA, 20 bp, Artificial Sequence
  Primer
caatatattctgcctccccg

SEQ ID NO: 17 - DNA, 20 bp, Artificial Sequence
  Primer
gtgctgttgttcccaagaca

SEQ ID NO: 18 - DNA, 20 bp, Artificial Sequence
  Primer
gccatcatcacagagctcac

SEQ ID NO: 19 - DNA, 25 bp, Artificial Sequence
  Primer
cgcgtagtgatgccatgtaactgaa

SEQ ID NO: 20 - DNA, 25 bp, Artificial Sequence
  Primer
cgcttcgatcccaagaaggaatcaa

SEQ ID NO: 21 - DNA, 18 bp, Artificial Sequence
  Primer
cctggcatgcaagtgtga

SEQ ID NO: 22 - DNA, 19 bp, Artificial Sequence
  Primer
cgaatggtcacccgagttt

SEQ ID NO: 23 - DNA, 19 bp, Artificial Sequence
  Primer
tcagagcactgggacgaag

SEQ ID NO: 24 - DNA, 18 bp, Artificial Sequence
  Primer
cccaacacctccaaccat

SEQ ID NO: 25 - DNA, 27 bp, Artificial Sequence
  Primer
gcacagggaagtcacagatgtatgtgc

SEQ ID NO: 26 - DNA, 24 bp, Artificial Sequence
  Primer
ccactggtcacgttcaggatgaag

SEQ ID NO: 27 - DNA, 25 bp, Artificial Sequence
  Primer
gggtacccagttaaattttcatttc

SEQ ID NO: 28 - DNA, 26 bp, Artificial Sequence
  Primer
caagtttcaaccagcaagaaattact

SEQ ID NO: 29 - DNA, 20 bp, Artificial Sequence
  Primer
gtggcacagaattgctctca

SEQ ID NO: 30 - DNA, 20 bp, Artificial Sequence
  Primer
tcaccctcaaacacctcctc

SEQ ID NO: 31 - DNA, 19 bp, Artificial Sequence
  Primer
gaaggtgaaggtcggagtc

SEQ ID NO: 32 - DNA, 20 bp, Artificial Sequence
  Primer
gaagatggtgatgggatttc

SEQ ID NO: 33 - DNA, 18 bp, Artificial Sequence
  Primer
cctggcatgcaagtgtga

SEQ ID NO: 34 - DNA, 19 bp, Artificial Sequence
  Primer
cgaatggtcacccgagttt

SEQ ID NO: 35 - DNA, 22 bp, Artificial Sequence
  Primer
gtgggatcgagacatgtaagca

SEQ ID NO: 36 - DNA, 19 bp, Artificial Sequence
  Primer
caatccaaatgcggcatct